European Patent Specification EP 3 316 850 B1, published September 11, 2024. Title: FUSOGENIC LIPOSOME-COATED POROUS SILICON NANOPARTICLES. Applicant: The Regents of the University of California. Application Not yet assigned. The sequence listing filed with the application follows.

SEQUENCE LISTING (1 sequence)

SEQ ID NO: 1 - protein, 33 aa, Rabies virus
CCGGYTIWMPENPRPGTPCDIFTNSRGKRASNG